European Patent Application EP 4 678 193 A1, published January 14, 2026. Title: RNAi agents having anti-obesity efficacy and combination therapy using the same. Applicant: 올릭스(주). Application WO. The sequence listing filed with the application follows.

SEQUENCE LISTING (6 sequences)

SEQ ID NO: 1 - RNA, 21 nt, synthetic construct
  source 1..21: mol_type = other RNA
tgagtaagcaatctggtcctt

SEQ ID NO: 2 - RNA, 19 nt, synthetic construct
  source 1..19: mol_type = other RNA
agatccagagctgcgccac

SEQ ID NO: 3 - RNA, 19 nt, synthetic construct
  source 1..19: mol_type = other RNA
tgatccagagctgcgccac

SEQ ID NO: 4 - RNA, 16 nt, synthetic construct
  source 1..16: mol_type = other RNA
ccagattgcttactca

SEQ ID NO: 5 - RNA, 16 nt, synthetic construct
  source 1..16: mol_type = other RNA
gcgcagctctggatct

SEQ ID NO: 6 - RNA, 16 nt, synthetic construct
  source 1..16: mol_type = other RNA
gcgcagctctggatca